European Patent Application EP 4 169 934 A1, published April 26, 2023. Title: MUTANT OF IMMUNOGLOBULIN DEGRADING ENZYME IDEE. Applicant: Shanghai Bao Pharmaceuticals Co., Ltd. The sequence listing filed with the application follows.

SEQUENCE LISTING (35 sequences)

SEQ ID NO: 1 - protein, 349 aa, Artificial Sequence
  IdeE full sequence
MKTIAYPNKPHSLSAGLLTAIAIFSLASSNITYADDYQRNATEAYAKEVPHQITSVWTKGVTPLTPEQFRYNNEDVIHAPYLAHQGWYDITKAFDGKDNLLCGAATAGNMLHWWFDQNKTEIEAYLSKHPEKQKIIFNNQELFDLKAAIDTKDSQTNSQLFNYFRDKAFPNLSARQLGVMPDLVLDMFINGYYLNVFKTQSTDVNRPYQDKDKRGGIFDAVFTRGDQTTLLTARHDLKNKGLNDISTIIKQELTEGRALALSHTYANVSISHVINLWGADFNAEGNLEAIYVTDSDANASIGMKKYFVGINAHRHVAISAKKIEGENIGAQVLGLFTLSSGKDIWQKLS

SEQ ID NO: 2 - protein, 315 aa, Artificial Sequence
  IdeE sequence
DDYQRNATEAYAKEVPHQITSVWTKGVTPLTPEQFRYNNEDVIHAPYLAHQGWYDITKAFDGKDNLLCGAATAGNMLHWWFDQNKTEIEAYLSKHPEKQKIIFNNQELFDLKAAIDTKDSQTNSQLFNYFRDKAFPNLSARQLGVMPDLVLDMFINGYYLNVFKTQSTDVNRPYQDKDKRGGIFDAVFTRGDQTTLLTARHDLKNKGLNDISTIIKQELTEGRALALSHTYANVSISHVINLWGADFNAEGNLEAIYVTDSDANASIGMKKYFVGINAHRHVAISAKKIEGENIGAQVLGLFTLSSGKDIWQKLS

SEQ ID NO: 3 - protein, 315 aa, Artificial Sequence
  T8D
DDYQRNADEAYAKEVPHQITSVWTKGVTPLTPEQFRYNNEDVIHAPYLAHQGWYDITKAFDGKDNLLCGAATAGNMLHWWFDQNKTEIEAYLSKHPEKQKIIFNNQELFDLKAAIDTKDSQTNSQLFNYFRDKAFPNLSARQLGVMPDLVLDMFINGYYLNVFKTQSTDVNRPYQDKDKRGGIFDAVFTRGDQTTLLTARHDLKNKGLNDISTIIKQELTEGRALALSHTYANVSISHVINLWGADFNAEGNLEAIYVTDSDANASIGMKKYFVGINAHRHVAISAKKIEGENIGAQVLGLFTLSSGKDIWQKLS

SEQ ID NO: 4 - protein, 315 aa, Artificial Sequence
  T8E
DDYQRNAEEAYAKEVPHQITSVWTKGVTPLTPEQFRYNNEDVIHAPYLAHQGWYDITKAFDGKDNLLCGAATAGNMLHWWFDQNKTEIEAYLSKHPEKQKIIFNNQELFDLKAAIDTKDSQTNSQLFNYFRDKAFPNLSARQLGVMPDLVLDMFINGYYLNVFKTQSTDVNRPYQDKDKRGGIFDAVFTRGDQTTLLTARHDLKNKGLNDISTIIKQELTEGRALALSHTYANVSISHVINLWGADFNAEGNLEAIYVTDSDANASIGMKKYFVGINAHRHVAISAKKIEGENIGAQVLGLFTLSSGKDIWQKLS

SEQ ID NO: 5 - protein, 315 aa, Artificial Sequence
  T8W
DDYQRNAWEAYAKEVPHQITSVWTKGVTPLTPEQFRYNNEDVIHAPYLAHQGWYDITKAFDGKDNLLCGAATAGNMLHWWFDQNKTEIEAYLSKHPEKQKIIFNNQELFDLKAAIDTKDSQTNSQLFNYFRDKAFPNLSARQLGVMPDLVLDMFINGYYLNVFKTQSTDVNRPYQDKDKRGGIFDAVFTRGDQTTLLTARHDLKNKGLNDISTIIKQELTEGRALALSHTYANVSISHVINLWGADFNAEGNLEAIYVTDSDANASIGMKKYFVGINAHRHVAISAKKIEGENIGAQVLGLFTLSSGKDIWQKLS

SEQ ID NO: 6 - protein, 315 aa, Artificial Sequence
  T8Y
DDYQRNAYEAYAKEVPHQITSVWTKGVTPLTPEQFRYNNEDVIHAPYLAHQGWYDITKAFDGKDNLLCGAATAGNMLHWWFDQNKTEIEAYLSKHPEKQKIIFNNQELFDLKAAIDTKDSQTNSQLFNYFRDKAFPNLSARQLGVMPDLVLDMFINGYYLNVFKTQSTDVNRPYQDKDKRGGIFDAVFTRGDQTTLLTARHDLKNKGLNDISTIIKQELTEGRALALSHTYANVSISHVINLWGADFNAEGNLEAIYVTDSDANASIGMKKYFVGINAHRHVAISAKKIEGENIGAQVLGLFTLSSGKDIWQKLS

SEQ ID NO: 7 - protein, 315 aa, Artificial Sequence
  A10K
DDYQRNATEKYAKEVPHQITSVWTKGVTPLTPEQFRYNNEDVIHAPYLAHQGWYDITKAFDGKDNLLCGAATAGNMLHWWFDQNKTEIEAYLSKHPEKQKIIFNNQELFDLKAAIDTKDSQTNSQLFNYFRDKAFPNLSARQLGVMPDLVLDMFINGYYLNVFKTQSTDVNRPYQDKDKRGGIFDAVFTRGDQTTLLTARHDLKNKGLNDISTIIKQELTEGRALALSHTYANVSISHVINLWGADFNAEGNLEAIYVTDSDANASIGMKKYFVGINAHRHVAISAKKIEGENIGAQVLGLFTLSSGKDIWQKLS

SEQ ID NO: 8 - protein, 315 aa, Artificial Sequence
  A10R
DDYQRNATERYAKEVPHQITSVWTKGVTPLTPEQFRYNNEDVIHAPYLAHQGWYDITKAFDGKDNLLCGAATAGNMLHWWFDQNKTEIEAYLSKHPEKQKIIFNNQELFDLKAAIDTKDSQTNSQLFNYFRDKAFPNLSARQLGVMPDLVLDMFINGYYLNVFKTQSTDVNRPYQDKDKRGGIFDAVFTRGDQTTLLTARHDLKNKGLNDISTIIKQELTEGRALALSHTYANVSISHVINLWGADFNAEGNLEAIYVTDSDANASIGMKKYFVGINAHRHVAISAKKIEGENIGAQVLGLFTLSSGKDIWQKLS

SEQ ID NO: 9 - protein, 315 aa, Artificial Sequence
  T24A
DDYQRNATEAYAKEVPHQITSVWAKGVTPLTPEQFRYNNEDVIHAPYLAHQGWYDITKAFDGKDNLLCGAATAGNMLHWWFDQNKTEIEAYLSKHPEKQKIIFNNQELFDLKAAIDTKDSQTNSQLFNYFRDKAFPNLSARQLGVMPDLVLDMFINGYYLNVFKTQSTDVNRPYQDKDKRGGIFDAVFTRGDQTTLLTARHDLKNKGLNDISTIIKQELTEGRALALSHTYANVSISHVINLWGADFNAEGNLEAIYVTDSDANASIGMKKYFVGINAHRHVAISAKKIEGENIGAQVLGLFTLSSGKDIWQKLS

SEQ ID NO: 10 - protein, 315 aa, Artificial Sequence
  T24G
DDYQRNATEAYAKEVPHQITSVWGKGVTPLTPEQFRYNNEDVIHAPYLAHQGWYDITKAFDGKDNLLCGAATAGNMLHWWFDQNKTEIEAYLSKHPEKQKIIFNNQELFDLKAAIDTKDSQTNSQLFNYFRDKAFPNLSARQLGVMPDLVLDMFINGYYLNVFKTQSTDVNRPYQDKDKRGGIFDAVFTRGDQTTLLTARHDLKNKGLNDISTIIKQELTEGRALALSHTYANVSISHVINLWGADFNAEGNLEAIYVTDSDANASIGMKKYFVGINAHRHVAISAKKIEGENIGAQVLGLFTLSSGKDIWQKLS

SEQ ID NO: 11 - protein, 315 aa, Artificial Sequence
  T24S
DDYQRNATEAYAKEVPHQITSVWSKGVTPLTPEQFRYNNEDVIHAPYLAHQGWYDITKAFDGKDNLLCGAATAGNMLHWWFDQNKTEIEAYLSKHPEKQKIIFNNQELFDLKAAIDTKDSQTNSQLFNYFRDKAFPNLSARQLGVMPDLVLDMFINGYYLNVFKTQSTDVNRPYQDKDKRGGIFDAVFTRGDQTTLLTARHDLKNKGLNDISTIIKQELTEGRALALSHTYANVSISHVINLWGADFNAEGNLEAIYVTDSDANASIGMKKYFVGINAHRHVAISAKKIEGENIGAQVLGLFTLSSGKDIWQKLS

SEQ ID NO: 12 - protein, 315 aa, Artificial Sequence
  A59I
DDYQRNATEAYAKEVPHQITSVWTKGVTPLTPEQFRYNNEDVIHAPYLAHQGWYDITKIFDGKDNLLCGAATAGNMLHWWFDQNKTEIEAYLSKHPEKQKIIFNNQELFDLKAAIDTKDSQTNSQLFNYFRDKAFPNLSARQLGVMPDLVLDMFINGYYLNVFKTQSTDVNRPYQDKDKRGGIFDAVFTRGDQTTLLTARHDLKNKGLNDISTIIKQELTEGRALALSHTYANVSISHVINLWGADFNAEGNLEAIYVTDSDANASIGMKKYFVGINAHRHVAISAKKIEGENIGAQVLGLFTLSSGKDIWQKLS

SEQ ID NO: 13 - protein, 315 aa, Artificial Sequence
  A59L
DDYQRNATEAYAKEVPHQITSVWTKGVTPLTPEQFRYNNEDVIHAPYLAHQGWYDITKLFDGKDNLLCGAATAGNMLHWWFDQNKTEIEAYLSKHPEKQKIIFNNQELFDLKAAIDTKDSQTNSQLFNYFRDKAFPNLSARQLGVMPDLVLDMFINGYYLNVFKTQSTDVNRPYQDKDKRGGIFDAVFTRGDQTTLLTARHDLKNKGLNDISTIIKQELTEGRALALSHTYANVSISHVINLWGADFNAEGNLEAIYVTDSDANASIGMKKYFVGINAHRHVAISAKKIEGENIGAQVLGLFTLSSGKDIWQKLS

SEQ ID NO: 14 - protein, 315 aa, Artificial Sequence
  A59V
DDYQRNATEAYAKEVPHQITSVWTKGVTPLTPEQFRYNNEDVIHAPYLAHQGWYDITKVFDGKDNLLCGAATAGNMLHWWFDQNKTEIEAYLSKHPEKQKIIFNNQELFDLKAAIDTKDSQTNSQLFNYFRDKAFPNLSARQLGVMPDLVLDMFINGYYLNVFKTQSTDVNRPYQDKDKRGGIFDAVFTRGDQTTLLTARHDLKNKGLNDISTIIKQELTEGRALALSHTYANVSISHVINLWGADFNAEGNLEAIYVTDSDANASIGMKKYFVGINAHRHVAISAKKIEGENIGAQVLGLFTLSSGKDIWQKLS

SEQ ID NO: 15 - protein, 315 aa, Artificial Sequence
  E97D
DDYQRNATEAYAKEVPHQITSVWTKGVTPLTPEQFRYNNEDVIHAPYLAHQGWYDITKAFDGKDNLLCGAATAGNMLHWWFDQNKTEIEAYLSKHPDKQKIIFNNQELFDLKAAIDTKDSQTNSQLFNYFRDKAFPNLSARQLGVMPDLVLDMFINGYYLNVFKTQSTDVNRPYQDKDKRGGIFDAVFTRGDQTTLLTARHDLKNKGLNDISTIIKQELTEGRALALSHTYANVSISHVINLWGADFNAEGNLEAIYVTDSDANASIGMKKYFVGINAHRHVAISAKKIEGENIGAQVLGLFTLSSGKDIWQKLS

SEQ ID NO: 16 - protein, 315 aa, Artificial Sequence
  R280H
DDYQRNATEAYAKEVPHQITSVWTKGVTPLTPEQFRYNNEDVIHAPYLAHQGWYDITKAFDGKDNLLCGAATAGNMLHWWFDQNKTEIEAYLSKHPEKQKIIFNNQELFDLKAAIDTKDSQTNSQLFNYFRDKAFPNLSARQLGVMPDLVLDMFINGYYLNVFKTQSTDVNRPYQDKDKRGGIFDAVFTRGDQTTLLTARHDLKNKGLNDISTIIKQELTEGRALALSHTYANVSISHVINLWGADFNAEGNLEAIYVTDSDANASIGMKKYFVGINAHHHVAISAKKIEGENIGAQVLGLFTLSSGKDIWQKLS

SEQ ID NO: 17 - protein, 315 aa, Artificial Sequence
  R280K
DDYQRNATEAYAKEVPHQITSVWTKGVTPLTPEQFRYNNEDVIHAPYLAHQGWYDITKAFDGKDNLLCGAATAGNMLHWWFDQNKTEIEAYLSKHPEKQKIIFNNQELFDLKAAIDTKDSQTNSQLFNYFRDKAFPNLSARQLGVMPDLVLDMFINGYYLNVFKTQSTDVNRPYQDKDKRGGIFDAVFTRGDQTTLLTARHDLKNKGLNDISTIIKQELTEGRALALSHTYANVSISHVINLWGADFNAEGNLEAIYVTDSDANASIGMKKYFVGINAHKHVAISAKKIEGENIGAQVLGLFTLSSGKDIWQKLS

SEQ ID NO: 18 - protein, 300 aa, Artificial Sequence
  WT_del15
PHQITSVWTKGVTPLTPEQFRYNNEDVIHAPYLAHQGWYDITKAFDGKDNLLCGAATAGNMLHWWFDQNKTEIEAYLSKHPEKQKIIFNNQELFDLKAAIDTKDSQTNSQLFNYFRDKAFPNLSARQLGVMPDLVLDMFINGYYLNVFKTQSTDVNRPYQDKDKRGGIFDAVFTRGDQTTLLTARHDLKNKGLNDISTIIKQELTEGRALALSHTYANVSISHVINLWGADFNAEGNLEAIYVTDSDANASIGMKKYFVGINAHRHVAISAKKIEGENIGAQVLGLFTLSSGKDIWQKLS

SEQ ID NO: 19 - protein, 299 aa, Artificial Sequence
  WT_del16
HQITSVWTKGVTPLTPEQFRYNNEDVIHAPYLAHQGWYDITKAFDGKDNLLCGAATAGNMLHWWFDQNKTEIEAYLSKHPEKQKIIFNNQELFDLKAAIDTKDSQTNSQLFNYFRDKAFPNLSARQLGVMPDLVLDMFINGYYLNVFKTQSTDVNRPYQDKDKRGGIFDAVFTRGDQTTLLTARHDLKNKGLNDISTIIKQELTEGRALALSHTYANVSISHVINLWGADFNAEGNLEAIYVTDSDANASIGMKKYFVGINAHRHVAISAKKIEGENIGAQVLGLFTLSSGKDIWQKLS

SEQ ID NO: 20 - protein, 298 aa, Artificial Sequence
  WT_del17
QITSVWTKGVTPLTPEQFRYNNEDVIHAPYLAHQGWYDITKAFDGKDNLLCGAATAGNMLHWWFDQNKTEIEAYLSKHPEKQKIIFNNQELFDLKAAIDTKDSQTNSQLFNYFRDKAFPNLSARQLGVMPDLVLDMFINGYYLNVFKTQSTDVNRPYQDKDKRGGIFDAVFTRGDQTTLLTARHDLKNKGLNDISTIIKQELTEGRALALSHTYANVSISHVINLWGADFNAEGNLEAIYVTDSDANASIGMKKYFVGINAHRHVAISAKKIEGENIGAQVLGLFTLSSGKDIWQKLS

SEQ ID NO: 21 - protein, 297 aa, Artificial Sequence
  WT_del18
ITSVWTKGVTPLTPEQFRYNNEDVIHAPYLAHQGWYDITKAFDGKDNLLCGAATAGNMLHWWFDQNKTEIEAYLSKHPEKQKIIFNNQELFDLKAAIDTKDSQTNSQLFNYFRDKAFPNLSARQLGVMPDLVLDMFINGYYLNVFKTQSTDVNRPYQDKDKRGGIFDAVFTRGDQTTLLTARHDLKNKGLNDISTIIKQELTEGRALALSHTYANVSISHVINLWGADFNAEGNLEAIYVTDSDANASIGMKKYFVGINAHRHVAISAKKIEGENIGAQVLGLFTLSSGKDIWQKLS

SEQ ID NO: 22 - protein, 296 aa, Artificial Sequence
  WT_del19
TSVWTKGVTPLTPEQFRYNNEDVIHAPYLAHQGWYDITKAFDGKDNLLCGAATAGNMLHWWFDQNKTEIEAYLSKHPEKQKIIFNNQELFDLKAAIDTKDSQTNSQLFNYFRDKAFPNLSARQLGVMPDLVLDMFINGYYLNVFKTQSTDVNRPYQDKDKRGGIFDAVFTRGDQTTLLTARHDLKNKGLNDISTIIKQELTEGRALALSHTYANVSISHVINLWGADFNAEGNLEAIYVTDSDANASIGMKKYFVGINAHRHVAISAKKIEGENIGAQVLGLFTLSSGKDIWQKLS

SEQ ID NO: 23 - protein, 310 aa, Artificial Sequence
  WT_delC5
DDYQRNATEAYAKEVPHQITSVWTKGVTPLTPEQFRYNNEDVIHAPYLAHQGWYDITKAFDGKDNLLCGAATAGNMLHWWFDQNKTEIEAYLSKHPEKQKIIFNNQELFDLKAAIDTKDSQTNSQLFNYFRDKAFPNLSARQLGVMPDLVLDMFINGYYLNVFKTQSTDVNRPYQDKDKRGGIFDAVFTRGDQTTLLTARHDLKNKGLNDISTIIKQELTEGRALALSHTYANVSISHVINLWGADFNAEGNLEAIYVTDSDANASIGMKKYFVGINAHRHVAISAKKIEGENIGAQVLGLFTLSSGKDI

SEQ ID NO: 24 - protein, 305 aa, Artificial Sequence
  WT_delC10
DDYQRNATEAYAKEVPHQITSVWTKGVTPLTPEQFRYNNEDVIHAPYLAHQGWYDITKAFDGKDNLLCGAATAGNMLHWWFDQNKTEIEAYLSKHPEKQKIIFNNQELFDLKAAIDTKDSQTNSQLFNYFRDKAFPNLSARQLGVMPDLVLDMFINGYYLNVFKTQSTDVNRPYQDKDKRGGIFDAVFTRGDQTTLLTARHDLKNKGLNDISTIIKQELTEGRALALSHTYANVSISHVINLWGADFNAEGNLEAIYVTDSDANASIGMKKYFVGINAHRHVAISAKKIEGENIGAQVLGLFTLS

SEQ ID NO: 25 - protein, 297 aa, Artificial Sequence
  T24A_del18
ITSVWAKGVTPLTPEQFRYNNEDVIHAPYLAHQGWYDITKAFDGKDNLLCGAATAGNMLHWWFDQNKTEIEAYLSKHPEKQKIIFNNQELFDLKAAIDTKDSQTNSQLFNYFRDKAFPNLSARQLGVMPDLVLDMFINGYYLNVFKTQSTDVNRPYQDKDKRGGIFDAVFTRGDQTTLLTARHDLKNKGLNDISTIIKQELTEGRALALSHTYANVSISHVINLWGADFNAEGNLEAIYVTDSDANASIGMKKYFVGINAHRHVAISAKKIEGENIGAQVLGLFTLSSGKDIWQKLS

SEQ ID NO: 26 - protein, 297 aa, Artificial Sequence
  A59L_del18
ITSVWTKGVTPLTPEQFRYNNEDVIHAPYLAHQGWYDITKLFDGKDNLLCGAATAGNMLHWWFDQNKTEIEAYLSKHPEKQKIIFNNQELFDLKAAIDTKDSQTNSQLFNYFRDKAFPNLSARQLGVMPDLVLDMFINGYYLNVFKTQSTDVNRPYQDKDKRGGIFDAVFTRGDQTTLLTARHDLKNKGLNDISTIIKQELTEGRALALSHTYANVSISHVINLWGADFNAEGNLEAIYVTDSDANASIGMKKYFVGINAHRHVAISAKKIEGENIGAQVLGLFTLSSGKDIWQKLS

SEQ ID NO: 27 - protein, 297 aa, Artificial Sequence
  A59V_del18
ITSVWTKGVTPLTPEQFRYNNEDVIHAPYLAHQGWYDITKVFDGKDNLLCGAATAGNMLHWWFDQNKTEIEAYLSKHPEKQKIIFNNQELFDLKAAIDTKDSQTNSQLFNYFRDKAFPNLSARQLGVMPDLVLDMFINGYYLNVFKTQSTDVNRPYQDKDKRGGIFDAVFTRGDQTTLLTARHDLKNKGLNDISTIIKQELTEGRALALSHTYANVSISHVINLWGADFNAEGNLEAIYVTDSDANASIGMKKYFVGINAHRHVAISAKKIEGENIGAQVLGLFTLSSGKDIWQKLS

SEQ ID NO: 28 - protein, 297 aa, Artificial Sequence
  E97D_del18
ITSVWTKGVTPLTPEQFRYNNEDVIHAPYLAHQGWYDITKAFDGKDNLLCGAATAGNMLHWWFDQNKTEIEAYLSKHPDKQKIIFNNQELFDLKAAIDTKDSQTNSQLFNYFRDKAFPNLSARQLGVMPDLVLDMFINGYYLNVFKTQSTDVNRPYQDKDKRGGIFDAVFTRGDQTTLLTARHDLKNKGLNDISTIIKQELTEGRALALSHTYANVSISHVINLWGADFNAEGNLEAIYVTDSDANASIGMKKYFVGINAHRHVAISAKKIEGENIGAQVLGLFTLSSGKDIWQKLS

SEQ ID NO: 29 - protein, 297 aa, Artificial Sequence
  R280H_del18
ITSVWTKGVTPLTPEQFRYNNEDVIHAPYLAHQGWYDITKAFDGKDNLLCGAATAGNMLHWWFDQNKTEIEAYLSKHPEKQKIIFNNQELFDLKAAIDTKDSQTNSQLFNYFRDKAFPNLSARQLGVMPDLVLDMFINGYYLNVFKTQSTDVNRPYQDKDKRGGIFDAVFTRGDQTTLLTARHDLKNKGLNDISTIIKQELTEGRALALSHTYANVSISHVINLWGADFNAEGNLEAIYVTDSDANASIGMKKYFVGINAHHHVAISAKKIEGENIGAQVLGLFTLSSGKDIWQKLS

SEQ ID NO: 30 - protein, 292 aa, Artificial Sequence
  E97D_del18_delC5
ITSVWTKGVTPLTPEQFRYNNEDVIHAPYLAHQGWYDITKAFDGKDNLLCGAATAGNMLHWWFDQNKTEIEAYLSKHPDKQKIIFNNQELFDLKAAIDTKDSQTNSQLFNYFRDKAFPNLSARQLGVMPDLVLDMFINGYYLNVFKTQSTDVNRPYQDKDKRGGIFDAVFTRGDQTTLLTARHDLKNKGLNDISTIIKQELTEGRALALSHTYANVSISHVINLWGADFNAEGNLEAIYVTDSDANASIGMKKYFVGINAHRHVAISAKKIEGENIGAQVLGLFTLSSGKDI

SEQ ID NO: 31 - protein, 287 aa, Artificial Sequence
  E97D_del18_delC10
ITSVWTKGVTPLTPEQFRYNNEDVIHAPYLAHQGWYDITKAFDGKDNLLCGAATAGNMLHWWFDQNKTEIEAYLSKHPDKQKIIFNNQELFDLKAAIDTKDSQTNSQLFNYFRDKAFPNLSARQLGVMPDLVLDMFINGYYLNVFKTQSTDVNRPYQDKDKRGGIFDAVFTRGDQTTLLTARHDLKNKGLNDISTIIKQELTEGRALALSHTYANVSISHVINLWGADFNAEGNLEAIYVTDSDANASIGMKKYFVGINAHRHVAISAKKIEGENIGAQVLGLFTLS

SEQ ID NO: 32 - protein, 292 aa, Artificial Sequence
  A59V_del18_delC5
ITSVWTKGVTPLTPEQFRYNNEDVIHAPYLAHQGWYDITKVFDGKDNLLCGAATAGNMLHWWFDQNKTEIEAYLSKHPEKQKIIFNNQELFDLKAAIDTKDSQTNSQLFNYFRDKAFPNLSARQLGVMPDLVLDMFINGYYLNVFKTQSTDVNRPYQDKDKRGGIFDAVFTRGDQTTLLTARHDLKNKGLNDISTIIKQELTEGRALALSHTYANVSISHVINLWGADFNAEGNLEAIYVTDSDANASIGMKKYFVGINAHRHVAISAKKIEGENIGAQVLGLFTLSSGKDI

SEQ ID NO: 33 - protein, 292 aa, Artificial Sequence
  A59L_del18_delC5
ITSVWTKGVTPLTPEQFRYNNEDVIHAPYLAHQGWYDITKLFDGKDNLLCGAATAGNMLHWWFDQNKTEIEAYLSKHPEKQKIIFNNQELFDLKAAIDTKDSQTNSQLFNYFRDKAFPNLSARQLGVMPDLVLDMFINGYYLNVFKTQSTDVNRPYQDKDKRGGIFDAVFTRGDQTTLLTARHDLKNKGLNDISTIIKQELTEGRALALSHTYANVSISHVINLWGADFNAEGNLEAIYVTDSDANASIGMKKYFVGINAHRHVAISAKKIEGENIGAQVLGLFTLSSGKDI

SEQ ID NO: 34 - protein, 292 aa, Artificial Sequence
  R280H_del18_delC5
ITSVWTKGVTPLTPEQFRYNNEDVIHAPYLAHQGWYDITKAFDGKDNLLCGAATAGNMLHWWFDQNKTEIEAYLSKHPEKQKIIFNNQELFDLKAAIDTKDSQTNSQLFNYFRDKAFPNLSARQLGVMPDLVLDMFINGYYLNVFKTQSTDVNRPYQDKDKRGGIFDAVFTRGDQTTLLTARHDLKNKGLNDISTIIKQELTEGRALALSHTYANVSISHVINLWGADFNAEGNLEAIYVTDSDANASIGMKKYFVGINAHHHVAISAKKIEGENIGAQVLGLFTLSSGKDI

SEQ ID NO: 35 - protein, 315 aa, Artificial Sequence
  A59V/E97D/R280H
DDYQRNATEAYAKEVPHQITSVWTKGVTPLTPEQFRYNNEDVIHAPYLAHQGWYDITKVFDGKDNLLCGAATAGNMLHWWFDQNKTEIEAYLSKHPDKQKIIFNNQELFDLKAAIDTKDSQTNSQLFNYFRDKAFPNLSARQLGVMPDLVLDMFINGYYLNVFKTQSTDVNRPYQDKDKRGGIFDAVFTRGDQTTLLTARHDLKNKGLNDISTIIKQELTEGRALALSHTYANVSISHVINLWGADFNAEGNLEAIYVTDSDANASIGMKKYFVGINAHHHVAISAKKIEGENIGAQVLGLFTLSSGKDIWQKLS